European Patent Application EP 4 424 697 A2, published September 4, 2024. Title: ULTRA-PURE AGONISTS OF GUANYLATE CYCLASE C, METHOD OF MAKING AND USING SAME. Applicant: Bausch Health Ireland Limited. The sequence listing filed with the application follows.

SEQUENCE LISTING (252 sequences)

SEQ ID NO: 1 - protein, 16 aa, synthetic construct
  REGION 1..16: note = Chemically Synthesized
NDECELCVNVACTGCL

SEQ ID NO: 2 - protein, 15 aa, synthetic construct
  REGION 1..15: note = Chemically Synthesized
DECELCVNVACTGCL

SEQ ID NO: 3 - protein, 14 aa, synthetic construct
  REGION 1..14: note = Chemically Synthesized
DECELCVNVACTGC

SEQ ID NO: 4 - protein, 14 aa, synthetic construct
  REGION 1..14: note = Chemcially Synthesized
ECELCVNVACTGCL

SEQ ID NO: 5 - protein, 13 aa, synthetic construct
  REGION 1..13: note = Chemically Synthesized
ECELCVNVACTGC

SEQ ID NO: 6 - protein, 13 aa, synthetic construct
  REGION 1..13: note = Chemically Synthesized
CELCVNVACTGCL

SEQ ID NO: 7 - protein, 12 aa, synthetic construct
  REGION 1..12: note = Chemically Synthesized
CELCVNVACTGC

SEQ ID NO: 8 - protein, 16 aa, synthetic construct
  REGION 1..16: note = Chemically Synthesized
  SITE 16: note = MISC_FEATURE - wherein LEU is a D amino acid
NDECELCVNVACTGCL

SEQ ID NO: 9 - protein, 16 aa, synthetic construct
  REGION 1..16: note = Chemically Synthesized
  SITE 1: note = MISC_FEATURE - wherein ASN is a D amino acid
  SITE 16: note = MISC_FEATURE - wherein LEU is a D amino acid
NDECELCVNVACTGCL

SEQ ID NO: 10 - protein, 16 aa, synthetic construct
  REGION 1..16: note = Chemically Synthesized
  SITE 1: note = MISC_FEATURE - wherein ASN is a D amino acid
  SITE 2: note = MISC_FEATURE - wherein ASP is a D amino acid
  SITE 16: note = MISC_FEATURE - wherein LEU is a D amino acid
NDECELCVNVACTGCL

SEQ ID NO: 11 - protein, 16 aa, synthetic construct
  REGION 1..16: note = Chemically Synthesized
  SITE 1: note = MISC_FEATURE - wherein ASN is a D amino acid
  SITE 2: note = MISC_FEATURE - wherein ASP is a D amino acid
  SITE 3: note = MISC_FEATURE - wherein GLU is a D amino acid
  SITE 16: note = MISC_FEATURE - wherein LEU is a D amino acid
NDECELCVNVACTGCL

SEQ ID NO: 12 - protein, 16 aa, synthetic construct
  REGION 1..16: note = Chemically Synthesized
  SITE 1: note = MISC_FEATURE - wherein ASN is a D amino acid
NDECELCVNVACTGCL

SEQ ID NO: 13 - protein, 16 aa, synthetic construct
  REGION 1..16: note = Chemically Synthesized
  SITE 1: note = MISC_FEATURE - wherein ASN is a D amino acid
  SITE 6: note = MISC_FEATURE - wherein LEU is a D amino acid
  SITE 16: note = MISC_FEATURE - wherein LEU is a D amino acid
NDECELCVNVACTGCL

SEQ ID NO: 14 - protein, 15 aa, synthetic construct
  REGION 1..15: note = Chemically Synthesized
NDECELCVNVACTGC

SEQ ID NO: 15 - protein, 16 aa, synthetic construct
  REGION 1..16: note = Chemically Synthesized
  SITE 1: note = MISC_FEATURE - wherein ASN at position 1 is attached to polyethylene glycol
  SITE 16: note = MISC_FEATURE - wherein LEU is a D amino acid
  SITE 16: note = MISC_FEATURE - wherein LEU at position 16 is attached to polyethylene glycol
NDECELCVNVACTGCL

SEQ ID NO: 16 - protein, 16 aa, synthetic construct
  REGION 1..16: note = Chemically Synthesized
  SITE 1: note = MISC_FEATURE - wherein ASN at position 1 is attached to polyethylene glycol
  SITE 1: note = MISC_FEATURE - wherein ASN is a D amino acid
  SITE 16: note = MISC_FEATURE - wherein LEU is a D amino acid
  SITE 16: note = MISC_FEATURE - wherein LEU at position 16 is attached to polyethylene glycol
NDECELCVNVACTGCL

SEQ ID NO: 17 - protein, 16 aa, synthetic construct
  REGION 1..16: note = Chemically Synthesized
  SITE 1: note = MISC_FEATURE - wherein ASN at position 1 is attached to polyethylene glycol
  SITE 1: note = MISC_FEATURE - wherein ASN is a D amino acid
  SITE 2: note = MISC_FEATURE - wherein ASP is a D amino acid
  SITE 16: note = MISC_FEATURE - wherein LEU is a D amino acid
  SITE 16: note = MISC_FEATURE - wherein LEU at position 16 is attached to polyethylene glycol
NDECELCVNVACTGCL

SEQ ID NO: 18 - protein, 16 aa, synthetic construct
  REGION 1..16: note = Chemically Synthesized
  SITE 1: note = MISC_FEATURE - wherein ASN is a D amino acid
  SITE 16: note = MISC_FEATURE - wherein LEU at position 16 is attached to polyethylene glycol
  SITE 16: note = MISC_FEATURE - wherein LEU is a D amino acid
NDECELCVNVACTGCL

SEQ ID NO: 19 - protein, 16 aa, synthetic construct
  REGION 1..16: note = Chemically Synthesized
  SITE 1: note = MISC_FEATURE - wherein ASN at position 1 is attached to polyethylene glycol
  SITE 16: note = MISC_FEATURE - wherein LEU is a D amino acid
NDECELCVNVACTGCL

SEQ ID NO: 20 - protein, 16 aa, synthetic construct
  REGION 1..16: note = Chemically Synthesized
  SITE 1: note = MISC_FEATURE - wherein ASN at position 1 is attached to polyethylene glycol
  SITE 1: note = MISC_FEATURE - wherein ASN is a D amino acid
  SITE 16: note = MISC_FEATURE - wherein LEU is a D amino acid
NDECELCVNVACTGCL

SEQ ID NO: 21 - protein, 16 aa, synthetic construct
  REGION 1..16: note = Chemically Synthesized
  SITE 16: note = MISC_FEATURE - wherein LEU at position 16 is attached to polyethylene glycol
  SITE 16: note = MISC_FEATURE - wherein LEU is a D amino acid
NDECELCVNVACTGCL

SEQ ID NO: 22 - protein, 16 aa, synthetic construct
  REGION 1..16: note = Chemically Synthesized
  SITE 1: note = MISC_FEATURE - wherein ASN at position 1 is attached to polyethylene glycol
  SITE 1: note = MISC_FEATURE - wherein ASN is a D amino acid
  SITE 2: note = MISC_FEATURE - wherein ASP is a D amino acid
  SITE 3: note = MISC_FEATURE - wherein GLU is a D amino acid
  SITE 16: note = MISC_FEATURE - wherein LEU is a D amino acid
  SITE 16: note = MISC_FEATURE - wherein LEU at position 16 is attached to polyethylene glycol
NDECELCVNVACTGCL

SEQ ID NO: 23 - protein, 16 aa, synthetic construct
  REGION 1..16: note = Chemically Synthesized
  SITE 1: note = MISC_FEATURE - wherein ASN at position 1 is attached to polyethylene glycol
  SITE 1: note = MISC_FEATURE - wherein ASN is a D amino acid
  SITE 2: note = MISC_FEATURE - wherein ASP is a D amino acid
  SITE 3: note = MISC_FEATURE - wherein GLU is a D amino acid
  SITE 16: note = MISC_FEATURE - wherein LEU is a D amino acid
NDECELCVNVACTGCL

SEQ ID NO: 24 - protein, 16 aa, synthetic construct
  REGION 1..16: note = Chemically Synthesized
  SITE 1: note = MISC_FEATURE - wherein ASN is a D amino acid
  SITE 2: note = MISC_FEATURE - wherein ASP is a D amino acid
  SITE 3: note = MISC_FEATURE - wherein GLU is a D amino acid
  SITE 16: note = MISC_FEATURE - wherein LEU at position 16 is attached to polyethylene glycol
  SITE 16: note = MISC_FEATURE - wherein LEU is a D amino acid
NDECELCVNVACTGCL

SEQ ID NO: 25 - protein, 16 aa, synthetic construct
  REGION 1..16: note = Chemically Synthesized
  SITE 1: note = MISC_FEATURE - wherein ASN is a D amino acid
  SITE 2: note = MISC_FEATURE - wherein ASP is a D amino acid
  SITE 16: note = MISC_FEATURE - wherein LEU at position 16 is attached to polyethylene glycol
  SITE 16: note = MISC_FEATURE - wherein LEU is a D amino acid
NDECELCVNVACTGCL

SEQ ID NO: 26 - protein, 16 aa, synthetic construct
  REGION 1..16: note = Chemically Synthesized
  SITE 1: note = MISC_FEATURE - wherein ASN at position 1 is attached to polyethylene glycol
  SITE 1: note = MISC_FEATURE - wherein ASN is a D amino acid
  SITE 2: note = MISC_FEATURE - wherein ASP is a D amino acid
  SITE 16: note = MISC_FEATURE - wherein LEU is a D amino acid
NDECELCVNVACTGCL

SEQ ID NO: 27 - protein, 16 aa, synthetic construct
  REGION 1..16: note = Chemically Synthesized
  SITE 1: note = MISC_FEATURE - wherein ASN is a D amino acid
  SITE 16: note = MISC_FEATURE - wherein x is 3-(2-naphthyl)alanine
  SITE 16: note = MISC_FEATURE - wherein x is a D amino acid
NDECELCVNVACTGCX

SEQ ID NO: 28 - protein, 16 aa, synthetic construct
  REGION 1..16: note = Chemically Synthesized
  SITE 1: note = MISC_FEATURE - wherein ASN is a D amino acid
  SITE 8: note = MISC_FEATURE - wherein x at position 8 is alpha-amino isobutyric acid
  SITE 10: note = MISC_FEATURE - wherein x at position 10 is alpha-amino isobutyric acid
  SITE 16: note = MISC_FEATURE - wherein LEU is a D amino acid
NDECELCXNXACTGCL

SEQ ID NO: 29 - protein, 16 aa, synthetic construct
  REGION 1..16: note = Chemically Synthesized
  SITE 1: note = MISC_FEATURE - wherein ASN is a D amino acid
  SITE 7: note = MISC_FEATURE - wherein ASP at position 7 is attached to a Lactam bridge
  SITE 15: note = MISC_FEATURE - wherein x at position 15 is ornithine
  SITE 16: note = MISC_FEATURE - wherein LEU is a D amino acid
NDECELDVNVACTGXL

SEQ ID NO: 30 - protein, 16 aa, synthetic construct
  REGION 1..16: note = Chemically Synthesized
  SITE 1: note = MISC_FEATURE - wherein ASN is a D amino acid
  SITE 16: note = MISC_FEATURE - wherein LEU is a D amino acid
NDECEYCVNVACTGCL

SEQ ID NO: 31 - protein, 16 aa, synthetic construct
  REGION 1..16: note = Chemically Synthesized
  SITE 1: note = MISC_FEATURE - wherein ASN is a D amino acid
  SITE 16: note = MISC_FEATURE - wherein LEU is a D amino acid
NDECESCVNVACTGCL

SEQ ID NO: 32 - protein, 16 aa, synthetic construct
  REGION 1..16: note = Chemically Synthesized
  SITE 1: note = MISC_FEATURE - wherein ASN at position 1 is attached to polyethylene glycol
  SITE 1: note = MISC_FEATURE - wherein ASN is a D amino acid
  SITE 16: note = MISC_FEATURE - wherein LEU is a D amino acid
  SITE 16: note = MISC_FEATURE - wherein LEU at position 16 is attached to polyethylene glycol
NDECEYCVNVACTGCL

SEQ ID NO: 33 - protein, 16 aa, synthetic construct
  REGION 1..16: note = Chemically Synthesized
  SITE 1: note = MISC_FEATURE - wherein ASN at position 1 is attached to polyethylene glycol
  SITE 1: note = MISC_FEATURE - wherein ASN is a D amino acid
  SITE 16: note = MISC_FEATURE - wherein LEU is a D amino acid
NDECEYCVNVACTGCL

SEQ ID NO: 34 - protein, 16 aa, synthetic construct
  REGION 1..16: note = Chemically Synthesized
  SITE 1: note = MISC_FEATURE - wherein ASN is a D amino acid
  SITE 16: note = MISC_FEATURE - wherein LEU at position 16 is attached to polyethylene glycol
  SITE 16: note = MISC_FEATURE - wherein LEU is a D amino acid
NDECEYCVNVACTGCL

SEQ ID NO: 35 - protein, 16 aa, synthetic construct
  REGION 1..16: note = Chemically Synthesized
  SITE 1: note = MISC_FEATURE - wherein ASN at position 1 is attached to polyethylene glycol
  SITE 1: note = MISC_FEATURE - wherein ASN is a D amino acid
  SITE 16: note = MISC_FEATURE - wherein LEU is a D amino acid
  SITE 16: note = MISC_FEATURE - wherein LEU at position 16 is attached to polyethylene glycol
NDECESCVNVACTGCL

SEQ ID NO: 36 - protein, 16 aa, synthetic construct
  REGION 1..16: note = Chemically Synthesized
  SITE 1: note = MISC_FEATURE - wherein ASN at position 1 is attached to polyethylene glycol
  SITE 1: note = MISC_FEATURE - wherein ASN is a D amino acid
  SITE 16: note = MISC_FEATURE - wherein LEU is a D amino acid
NDECESCVNVACTGCL

SEQ ID NO: 37 - protein, 16 aa, synthetic construct
  REGION 1..16: note = Chemically Synthesized
  SITE 1: note = MISC_FEATURE - wherein ASN is a D amino acid
  SITE 16: note = MISC_FEATURE - wherein LEU at position 16 is attached to polyethylene glycol
  SITE 16: note = MISC_FEATURE - wherein LEU is a D amino acid
NDECESCVNVACTGCL

SEQ ID NO: 38 - protein, 16 aa, synthetic construct
  REGION 1..16: note = Chemically Synthesized
NDECELCVNVACTGCS

SEQ ID NO: 39 - protein, 16 aa, synthetic construct
  REGION 1..16: note = Chemically Synthesized
  SITE 1: note = MISC_FEATURE - wherein ASN at position 1 is attached to polyethylene glycol
  SITE 16: note = MISC_FEATURE - wherein SER at position 16 is attached to polyethylene glycol
NDECELCVNVACTGCS

SEQ ID NO: 40 - protein, 16 aa, synthetic construct
  REGION 1..16: note = Chemically Synthesized
  SITE 1: note = MISC_FEATURE - wherein ASN at position 1 is attached to polyethylene glycol
NDECELCVNVACTGCS

SEQ ID NO: 41 - protein, 16 aa, synthetic construct
  REGION 1..16: note = Chemically Synthesized
  SITE 16: note = MISC_FEATURE - wherein SER at position 16 is attached to polyethylene glycol
NDECELCVNVACTGCS

SEQ ID NO: 42 - protein, 16 aa, synthetic construct
  REGION 1..16: note = Chemically Synthesized
  SITE 1: note = MISC_FEATURE - wherein ASN at position 1 is attached to polyethylene glycol
  SITE 16: note = MISC_FEATURE - wherein SER is a D amino acid
  SITE 16: note = MISC_FEATURE - wherein SER at position 16 is attached to polyethylene glycol
NDECELCVNVACTGCS

SEQ ID NO: 43 - protein, 16 aa, synthetic construct
  REGION 1..16: note = Chemically Synthesized
  SITE 1: note = MISC_FEATURE - wherein ASN at position 1 is attached to polyethylene glycol
  SITE 16: note = MISC_FEATURE - wherein SER is a D amino acid
NDECELCVNVACTGCS

SEQ ID NO: 44 - protein, 16 aa, synthetic construct
  REGION 1..16: note = Chemically Synthesized
  SITE 16: note = MISC_FEATURE - wherein SER at position 16 is attached to polyethylene glycol
  SITE 16: note = MISC_FEATURE - wherein SER is a D amino acid
NDECELCVNVACTGCS

SEQ ID NO: 45 - protein, 16 aa, synthetic construct
  REGION 1..16: note = Chemically Synthesized
  REGION 5..6: note = MISC_FEATURE - x is natural, unnatural, an analogue, L, D, or methylated amino acid or any combination
  REGION 8..11: note = MISC_FEATURE - x is natural, unnatural, an analogue, L, D, or methylated amino acid or any combination
  REGION 13..14: note = MISC_FEATURE - x is natural, unnatural, an analogue, L, D, or methylated amino acid or any combination
  SITE 16: note = MISC_FEATURE - x is natural, unnatural, an analogue, L, D, or methylated amino acid or any combination
NDECXXCXXXXCXXCX

SEQ ID NO: 46 - protein, 16 aa, synthetic construct
  REGION 1..16: note = Chemically Synthesized
  SITE 1: note = MISC_FEATURE - x is none or a natural, unnatural or an analogue amino acid, may be L, D, or a methylated amino acid, or any combination.
  SITE 2: note = MISC_FEATURE - x is none or a natural, unnatural or an analogue amino acid, may be L, D, or a methylated amino acid, or any combination.
  SITE 3: note = MISC_FEATURE - x is any natural, unnatural or an analogue amino acid, may be L, D, or a methylated amino acid, or any combination.
  REGION 5..6: note = MISC_FEATURE - x is natural, unnatural, analogue, L, D, or methylated amino acid or any combination
  REGION 8..11: note = MISC_FEATURE - x is natural, unnatural, analogue, L, D, or methylated amino acid or any combination
  REGION 13..14: note = MISC_FEATURE - x is natural, unnatural, analogue, L, D, or methylated amino acid or any combination
  SITE 16: note = MISC_FEATURE - x is none or one natural, unnatural or an analogue amino acid, may be L, D, or a methylated amino acid, or any combination
XXXCXXCXXXXCXXCX

SEQ ID NO: 47 - protein, 16 aa, synthetic construct
  REGION 1..16: note = Chemically Synthesized
  SITE 1: note = MISC_FEATURE - x is none or a natural, unnatural or an analogue amino acid, may be L, D, or a methylated amino acid or any combination thereof
  SITE 2: note = MISC_FEATURE - x is none or a natural, unnatural or an analogue amino acid, may be L, D, or a methylated amino acid or any combination thereof
  SITE 3: note = MISC_FEATURE - x is any natural, unnatural or an analogue amino acid, may be L, D, or a methylated amino acid or any combination thereof
  SITE 4: note = MISC_FEATURE - wherein x is a cysteine, penicillamine homocysteine, or 3-mercaptoproline
  SITE 6: note = MISC_FEATURE - x is natural, unnatural, analogue, L, D, or methylated amino acid or any combination
  SITE 7: note = MISC_FEATURE - wherein x is a cysteine, penicillamine homocysteine, or 3-mercaptoproline
  SITE 12: note = MISC_FEATURE - wherein x is a cysteine, penicillamine homocysteine, or 3-mercaptoproline
  SITE 15: note = MISC_FEATURE - wherein x is a cysteine, penicillamine homocysteine, or 3-mercaptoproline
  SITE 16: note = MISC_FEATURE - x is natural, unnatural or an analogue, zero or one residue in length, may be L, D, or a methylated amino acid or any combination thereof
XXXXEXXVNVAXTGXX

SEQ ID NO: 48 - skipped

SEQ ID NO: 49 - protein, 16 aa, synthetic construct
  REGION 1..16: note = Chemically Synthesized
  REGION 5..6: note = MISC_FEATURE - x is natural, unnatural, analogue, L, D, or methylated amino acid or any combination
  SITE 8: note = MISC_FEATURE - x is natural, unnatural, analogue, L, D, or methylated amino acid or any combination
  REGION 10..11: note = MISC_FEATURE - x is natural, unnatural, analogue, L, D, or methylated amino acid or any combination
  REGION 13..14: note = MISC_FEATURE - x is natural, unnatural, analogue, L, D, or methylated amino acid or any combination
  SITE 16: note = MISC_FEATURE - x is natural, unnatural, analogue, L, D, or methylated amino acid or any combination
NDDCXXCXNXXCXXCX

SEQ ID NO: 50 - protein, 16 aa, synthetic construct
  REGION 1..16: note = Chemically Synthesized
  SITE 1: note = MISC_FEATURE - wherein ASN is a D amino acid
  REGION 5..6: note = MISC_FEATURE - x is natural, unnatural, analogue, L, D, or methylated amino acid or any combination
  SITE 8: note = MISC_FEATURE - x is any natural, unnatural, analogue, L, D, or methylated amino acid or any combination
  REGION 10..11: note = MISC_FEATURE - x is natural, unnatural, analogue, L, D, or methylated amino acid or any combination
  REGION 13..14: note = MISC_FEATURE - x is natural, unnatural, analogue, L, D, or methylated amino acid or any combination
  SITE 16: note = MISC_FEATURE - x is natural, unnatural, analogue, L, D, or methylated amino acid or any combination
  SITE 16: note = MISC_FEATURE - wherein x is a D amino acid
NEECXXCXNXXCXXCX

SEQ ID NO: 51 - protein, 16 aa, synthetic construct
  REGION 1..16: note = Chemically Synthesized
  SITE 1: note = MISC_FEATURE - wherein ASN is a D amino acid
  SITE 2: note = MISC_FEATURE - wherein GLU is a D amino acid
  REGION 5..6: note = MISC_FEATURE - x is natural, unnatural, analogue, L, D, or methylated amino acid or any combination
  SITE 8: note = MISC_FEATURE - x is natural, unnatural, analogue, L, D, or methylated amino acid or any combination
  REGION 10..11: note = MISC_FEATURE - x is natural, unnatural, analogue, L, D, or methylated amino acid or any combination
  REGION 13..14: note = MISC_FEATURE - x is natural, unnatural, analogue, L, D, or methylated amino acid or any combination
  SITE 16: note = MISC_FEATURE - wherein x is a D amino acid
  SITE 16: note = MISC_FEATURE - x is natural, unnatural, analogue, L, D, or methylated amino acid or any combination
NEDCXXCXNXXCXXCX

SEQ ID NO: 52 - protein, 16 aa, synthetic construct
  REGION 1..16: note = Chemically Synthesized
  SITE 1: note = MISC_FEATURE - wherein ASN is a D amino acid
  SITE 2: note = MISC_FEATURE - wherein ASP is a D amino acid
  REGION 5..6: note = MISC_FEATURE - x is natural, unnatural, analogue, L, D, or methylated amino acid or any combination
  SITE 8: note = MISC_FEATURE - x is natural, unnatural, analogue, L, D, or methylated amino acid or any combination
  REGION 10..11: note = MISC_FEATURE - x is natural, unnatural, analogue, L, D, or methylated amino acid or any combination
  REGION 13..14: note = MISC_FEATURE - x is natural, unnatural, analogue, L, D, or methylated amino acid or any combination
  SITE 16: note = MISC_FEATURE - wherein x is a D amino acid
  SITE 16: note = MISC_FEATURE - x is natural, unnatural, analogue, L, D, or methylated amino acid or any combination
NDECXXCXNXXCXXCX

SEQ ID NO: 53 - protein, 16 aa, synthetic construct
  REGION 1..16: note = Chemically Synthesized
  SITE 1: note = MISC_FEATURE - wherein ASN is a D amino acid
  SITE 2: note = MISC_FEATURE - wherein ASP is a D amino acid
  SITE 3: note = MISC_FEATURE - wherein GLU is a D amino acid
  REGION 5..6: note = MISC_FEATURE - x is natural, unnatural, analogue, L, D, or methylated amino acid or any combination
  SITE 8: note = MISC_FEATURE - x is natural, unnatural, analogue, L, D, or methylated amino acid or any combination
  REGION 10..11: note = MISC_FEATURE - x is natural, unnatural, analogue, L, D, or methylated amino acid or any combination
  REGION 13..14: note = MISC_FEATURE - x is natural, unnatural, analogue, L, D, or methylated amino acid or any combination
  SITE 16: note = MISC_FEATURE - wherein x is a D amino acid
  SITE 16: note = MISC_FEATURE - x is natural, unnatural, analogue, L, D, or methylated amino acid or any combination
NDECXXCXYXXCXXCX

SEQ ID NO: 54 - protein, 16 aa, synthetic construct
  REGION 1..16: note = Chemically Synthesized
  SITE 1: note = MISC_FEATURE - wherein ASN is a D amino acid
  SITE 2: note = MISC_FEATURE - wherein GLU is a D amino acid
  SITE 3: note = MISC_FEATURE - wherein GLU is a D amino acid
  REGION 5..6: note = MISC_FEATURE - x is natural, unnatural, analogue, L, D, or methylated amino acid or any combination
  SITE 8: note = MISC_FEATURE - x is natural, unnatural, analogue, L, D, or methylated amino acid or any combination
  REGION 10..11: note = MISC_FEATURE - x is natural, unnatural, analogue, L, D, or methylated amino acid or any combination
  REGION 13..14: note = MISC_FEATURE - x is natural, unnatural, analogue, L, D, or methylated amino acid or any combination
  SITE 16: note = MISC_FEATURE - wherein x is a D amino acid
  SITE 16: note = MISC_FEATURE - x is natural, unnatural, analogue, L, D, or methylated amino acid or any combination
NEECXXCXYXXCXXCX

SEQ ID NO: 55 - protein, 14 aa, synthetic construct
  REGION 1..14: note = Chemically Synthesized
CCEYCCNPACTGCY

SEQ ID NO: 56 - protein, 13 aa, synthetic construct
  REGION 1..13: note = Chemically Synthesized
CCEYCCNPACTGC

SEQ ID NO: 57 - protein, 14 aa, synthetic construct
  REGION 1..14: note = Chemically Synthesized
  SITE 1: note = MISC_FEATURE - wherein CYS at position 1 is attached to polyethylene glycol
  SITE 14: note = MISC_FEATURE - wherein TYR at position 14 is attached to polyethylene glycol
CCEYCCNPACTGCY

SEQ ID NO: 58 - protein, 16 aa, synthetic construct
  REGION 1..16: note = Chemically Synthesized
NFCCESCCNPACTGCY

SEQ ID NO: 59 - protein, 16 aa, synthetic construct
  REGION 1..16: note = Chemically Synthesized
NFCCEFCCNPACTGCY

SEQ ID NO: 60 - protein, 14 aa, synthetic construct
  REGION 1..14: note = Chemically Synthesized
  SITE 14: note = MISC_FEATURE - wherein TYR is a D amino acid
CCEYCCNPACTGCY

SEQ ID NO: 61 - protein, 14 aa, synthetic construct
  REGION 1..14: note = Chemically Synthesized
  SITE 1: note = MISC_FEATURE - wherein CYS at position 1 is attached to polyethylene glycol
CCEYCCNPACTGCY

SEQ ID NO: 62 - protein, 16 aa, synthetic construct
  REGION 1..16: note = Chemically Synthesized
NFCCETCCNPACTGCY

SEQ ID NO: 63 - protein, 16 aa, synthetic construct
  REGION 1..16: note = Chemically Synthesized
  SITE 16: note = MISC_FEATURE - wherein TYR is a D amino acid
NFCCESCCNPACTGCY

SEQ ID NO: 64 - protein, 16 aa, synthetic construct
  REGION 1..16: note = Chemically Synthesized
  SITE 1: note = MISC_FEATURE - wherein ASN is a D amino acid
NFCCESCCNPACTGCY

SEQ ID NO: 65 - protein, 16 aa, synthetic construct
  REGION 1..16: note = Chemically Synthesized
  SITE 1: note = MISC_FEATURE - wherein ASN is a D amino acid
  SITE 16: note = MISC_FEATURE - wherein TYR is a D amino acid
NFCCESCCNPACTGCY

SEQ ID NO: 66 - protein, 16 aa, synthetic construct
  REGION 1..16: note = Chemically Synthesized
  SITE 16: note = MISC_FEATURE - wherein TYR is a D amino acid
NFCCETCCNPACTGCY

SEQ ID NO: 67 - protein, 16 aa, synthetic construct
  REGION 1..16: note = Chemically Synthesized
  SITE 1: note = MISC_FEATURE - wherein ASN is a D amino acid
NFCCETCCNPACTGCY

SEQ ID NO: 68 - protein, 16 aa, synthetic construct
  REGION 1..16: note = Chemically Synthesized
  SITE 1: note = MISC_FEATURE - wherein ASN is a D amino acid
  SITE 16: note = MISC_FEATURE - wherein TYR is a D amino acid
NFCCETCCNPACTGCY

SEQ ID NO: 69 - protein, 16 aa, synthetic construct
  REGION 1..16: note = Chemically Synthesized
  SITE 16: note = MISC_FEATURE - wherein TYR is a D amino acid
NFCCEFCCNPACTGCY

SEQ ID NO: 70 - protein, 16 aa, synthetic construct
  REGION 1..16: note = Chemically Synthesized
  SITE 1: note = MISC_FEATURE - wherein ASN is a D amino acid
NFCCEFCCNPACTGCY

SEQ ID NO: 71 - protein, 16 aa, synthetic construct
  REGION 1..16: note = Chemically Synthesized
  SITE 1: note = MISC_FEATURE - wherein ASN is a D amino acid
  SITE 16: note = MISC_FEATURE - wherein TYR is a D amino acid
NFCCEFCCNPACTGCY

SEQ ID NO: 72 - protein, 14 aa, synthetic construct
  REGION 1..14: note = Chemically Synthesized
  SITE 14: note = MISC_FEATURE - wherein TYR at position 14 is attached to polyethylene glycol
CCEYCCNPACTGCY

SEQ ID NO: 73 - protein, 13 aa, synthetic construct
  REGION 1..13: note = Chemically Synthesized
  SITE 1: note = MISC_FEATURE - wherein CYS at position 1 is attached to polyethylene glycol
  SITE 13: note = MISC_FEATURE - wherein CYS at position 13 is attached to polyethylene glycol
CCEYCCNPACTGC

SEQ ID NO: 74 - protein, 13 aa, synthetic construct
  REGION 1..13: note = Chemically Synthesized
  SITE 1: note = MISC_FEATURE - wherein CYS at position 1 is attached to polyethylene glycol
CCEYCCNPACTGC

SEQ ID NO: 75 - protein, 13 aa, synthetic construct
  REGION 1..13: note = Chemically Synthesized
  SITE 13: note = MISC_FEATURE - wherein CYS at position 13 is attached to polyethylene glycol
CCEYCCNPACTGC

SEQ ID NO: 76 - protein, 16 aa, synthetic construct
  REGION 1..16: note = Chemically Synthesized
  SITE 1: note = MISC_FEATURE - wherein ASN at position 1 is attached to polyethylene glycol
  SITE 16: note = MISC_FEATURE - wherein TYR at position 16 is attached to polyethylene glycol
NFCCESCCNPACTGCY

SEQ ID NO: 77 - protein, 16 aa, synthetic construct
  REGION 1..16: note = Chemically Synthesized
  SITE 1: note = MISC_FEATURE - wherein ASN at position 1 is attached to polyethylene glycol
NFCCESCCNPACTGCY

SEQ ID NO: 78 - protein, 16 aa, synthetic construct
  REGION 1..16: note = Chemically Synthesized
  SITE 16: note = MISC_FEATURE - wherein TYR at position 16 is attached to polyethylene glycol
NFCCESCCNPACTGCY

SEQ ID NO: 79 - protein, 16 aa, synthetic construct
  REGION 1..16: note = Chemically Synthesized
  SITE 1: note = MISC_FEATURE - wherein ASN at position 1 is attached to polyethylene glycol
  SITE 16: note = MISC_FEATURE - wherein TYR at position 16 is attached to polyethylene glycol
NFCCEFCCNPACTGCY

SEQ ID NO: 80 - protein, 16 aa, synthetic construct
  REGION 1..16: note = Chemically Synthesized
  SITE 1: note = MISC_FEATURE - wherein ASN at position 1 is attached to polyethylene glycol
NFCCEFCCNPACTGCY

SEQ ID NO: 81 - protein, 16 aa, synthetic construct
  REGION 1..16: note = Chemically Synthesized
  SITE 16: note = MISC_FEATURE - wherein TYR at position 16 is attached to polyethylene glycol
NFCCEFCCNPACTGCY

SEQ ID NO: 82 - protein, 16 aa, synthetic construct
  REGION 1..16: note = Chemically Synthesized
  SITE 1: note = MISC_FEATURE - wherein ASN at position 1 is attached to polyethylene glycol
  SITE 16: note = MISC_FEATURE - wherein TYR at position 16 is attached to polyethylene glycol
NFCCEYCCNPACTGCY

SEQ ID NO: 83 - protein, 16 aa, synthetic construct
  REGION 1..16: note = Chemically Synthesized
  SITE 1: note = MISC_FEATURE - wherein ASN at position 1 is attached to polyethylene glycol
NFCCEYCCNPACTGCY

SEQ ID NO: 84 - protein, 16 aa, synthetic construct
  REGION 1..16: note = Chemically Synthesized
  SITE 16: note = MISC_FEATURE - wherein TYR at position 16 is attached to polyethylene glycol
NFCCEYCCNPACTGCY

SEQ ID NO: 85 - protein, 14 aa, synthetic construct
  REGION 1..14: note = Chemically Synthesized
CCESCCNPACTGCY

SEQ ID NO: 86 - protein, 14 aa, synthetic construct
  REGION 1..14: note = Chemically Synthesized
CCEFCCNPACTGCY

SEQ ID NO: 87 - protein, 13 aa, synthetic construct
  REGION 1..13: note = Chemically Synthesized
CCESCCNPACTGC

SEQ ID NO: 88 - protein, 13 aa, synthetic construct
  REGION 1..13: note = Chemically Synthesized
CCEFCCNPACTGC

SEQ ID NO: 89 - protein, 14 aa, synthetic construct
  REGION 1..14: note = Chemically Synthesized
  REGION 1..2: note = MISC_FEATURE - wherein x is penicillamine
  REGION 5..6: note = MISC_FEATURE - wherein x is penicillamine
  SITE 10: note = MISC_FEATURE - wherein x is penicillamine
  SITE 13: note = MISC_FEATURE - wherein x is penicillamine
XXEYXXNPAXTGXY

SEQ ID NO: 90 - protein, 13 aa, synthetic construct
  REGION 1..13: note = Chemically Synthesized
  REGION 1..2: note = MISC_FEATURE - wherein x is penicillamine
  REGION 5..6: note = MISC_FEATURE - wherein x is penicillamine
  SITE 10: note = MISC_FEATURE - wherein x is penicillamine
  SITE 13: note = MISC_FEATURE - wherein x is penicillamine
XXEYXXNPAXTGX

SEQ ID NO: 91 - protein, 22 aa, synthetic construct
  REGION 1..22: note = Chemically Synthesized
  REGION 1..6: note = MISC_FEATURE - x is natural, unnatural, analogue, L, D, or methylated amino acid or any combination
  SITE 11: note = MISC_FEATURE - x is natural, unnatural, analogue, L, D, or methylated amino acid or any combination
  REGION 15..17: note = MISC_FEATURE - x is natural, unnatural, analogue, L, D, or methylated amino acid or any combination
  REGION 19..20: note = MISC_FEATURE - x is natural, unnatural, analogue, L, D, or methylated amino acid or any combination
  SITE 22: note = MISC_FEATURE - x is natural, unnatural, analogue, L, D, or methylated amino acid or any combination
XXXXXXNYCCXYCCXXXCXXCX

SEQ ID NO: 92 - protein, 22 aa, synthetic construct
  REGION 1..22: note = Chemically Synthesized
  REGION 1..6: note = MISC_FEATURE - x is natural, unnatural, analogue, L, D, or methylated amino acid or any combination
  SITE 11: note = MISC_FEATURE - x is natural, unnatural, analogue, L, D, or methylated amino acid or any combination
  REGION 15..17: note = MISC_FEATURE - x is natural, unnatural, analogue, L, D, or methylated amino acid or any combination
  REGION 19..20: note = MISC_FEATURE - x is natural, unnatural, analogue, L, D, or methylated amino acid or any combination
  SITE 22: note = MISC_FEATURE - x is natural, unnatural, analogue, L, D, or methylated amino acid or any combination
XXXXXXNFCCXFCCXXXCXXCX

SEQ ID NO: 93 - protein, 16 aa, synthetic construct
  REGION 1..16: note = Chemically Synthesized
  SITE 5: note = MISC_FEATURE - x is natural, unnatural, analogue, L, D, or methylated amino acid or any combination
  REGION 9..11: note = MISC_FEATURE - x is natural, unnatural, analogue, L, D, or methylated amino acid or any combination
  REGION 13..14: note = MISC_FEATURE - x is natural, unnatural, analogue, L, D, or methylated amino acid or any combination
  SITE 16: note = MISC_FEATURE - x is natural, unnatural, analogue, L, D, or methylated amino acid or any combination
NFCCXFCCXXXCXXCX

SEQ ID NO: 94 - protein, 16 aa, synthetic construct
  REGION 1..16: note = Chemically Synthesized
  SITE 3: note = MISC_FEATURE - wherein x is penicillamine
  SITE 5: note = MISC_FEATURE - x is natural, unnatural, analogue, L, D, or methylated amino acid or any combination
  SITE 8: note = MISC_FEATURE - wherein x is penicillamine
  REGION 9..11: note = MISC_FEATURE - x is natural, unnatural, analogue, L, D, or methylated amino acid or any combination
  REGION 13..14: note = MISC_FEATURE - x is natural, unnatural, analogue, L, D, or methylated amino acid or any combination
  SITE 16: note = MISC_FEATURE - x is natural, unnatural, analogue, L, D, or methylated amino acid or any combination
NFXCXFCXXXXCXXCX

SEQ ID NO: 95 - skipped

SEQ ID NO: 96 - protein, 14 aa, synthetic construct
  REGION 1..14: note = Chemically Synthesized
  REGION 1..2: note = MISC_FEATURE - wherein x is a cysteine, penicillamine homocysteine, or 3-mercaptoproline
  SITE 4: note = MISC_FEATURE - x is natural, unnatural, analogue, L, D, or methylated amino acid or any combination
  REGION 5..6: note = MISC_FEATURE - wherein x is a cysteine, penicillamine homocysteine, or 3-mercaptoproline
  SITE 10: note = MISC_FEATURE - wherein x is a cysteine, penicillamine homocysteine, or 3-mercaptoproline
  SITE 13: note = MISC_FEATURE - wherein x is a cysteine, penicillamine homocysteine, or 3-mercaptoproline
XXEXXXNPAXTGXY

SEQ ID NO: 97 - protein, 13 aa, synthetic construct
  REGION 1..13: note = Chemically Synthesized
  REGION 1..2: note = MISC_FEATURE - wherein x is a cysteine, penicillamine homocysteine, or 3-mercaptoproline
  SITE 4: note = MISC_FEATURE - x is natural, unnatural, analogue, L, D, or methylated amino acid or any combination
  REGION 5..6: note = MISC_FEATURE - wherein x is a cysteine, penicillamine homocysteine, or 3-mercaptoproline
  SITE 10: note = MISC_FEATURE - wherein x is a cysteine, penicillamine homocysteine, or 3-mercaptoproline
  SITE 13: note = MISC_FEATURE - wherein x is a cysteine, penicillamine homocysteine, or 3-mercaptoproline
XXEXXXNPAXTGX

SEQ ID NO: 98 - skipped

SEQ ID NO: 99 - protein, 16 aa, synthetic construct
  REGION 1..16: note = Chemically Synthesized
  SITE 1: note = MISC_FEATURE - wherein ASN is a D amino acid
  SITE 16: note = MISC_FEATURE - wherein LEU is a D amino acid
  SITE 16: note = MISC_FEATURE - wherein LEU is conjugated to an AMIDE
NDECELCVNVACTGCL

SEQ ID NO: 100 - protein, 16 aa, synthetic construct
  REGION 1..16: note = Chemically Synthesized
  SITE 1: note = MISC_FEATURE - wherein ASN is a D amino acid
  SITE 16: note = MISC_FEATURE - wherein SER is a D amino acid
NDECELCVNVACTGCS

SEQ ID NO: 101 - protein, 16 aa, synthetic construct
  REGION 1..16: note = Chemically Synthesized
  SITE 1: note = MISC_FEATURE - wherein ASN is a D amino acid
  SITE 16: note = MISC_FEATURE - wherein SER is a D amino acid
  SITE 16: note = MISC_FEATURE - wherein SER is conjugated to an AMIDE
NDECELCVNVACTGCS

SEQ ID NO: 102 - protein, 16 aa, synthetic construct
  REGION 1..16: note = Chemically Synthesized
  SITE 1: note = MISC_FEATURE - wherein ASN is a D amino acid
  SITE 16: note = MISC_FEATURE - wherein TYR is a D amino acid
NDECELCVNVACTGCY

SEQ ID NO: 103 - protein, 16 aa, synthetic construct
  REGION 1..16: note = Chemically Synthesized
  SITE 1: note = MISC_FEATURE - wherein ASN is a D amino acid
  SITE 16: note = MISC_FEATURE - wherein TYR is a D amino acid
  SITE 16: note = MISC_FEATURE - wherein TYR is conjugated to an AMIDE
NDECELCVNVACTGCY

SEQ ID NO: 104 - protein, 16 aa, synthetic construct
  REGION 1..16: note = Chemically Synthesized
  SITE 1: note = MISC_FEATURE - wherein GLU is conjugated to Py
  SITE 16: note = MISC_FEATURE - wherein LEU is conjugated to an AMIDE
  SITE 16: note = MISC_FEATURE - wherein LEU is a D amino acid
EDECELCVNVACTGCL

SEQ ID NO: 105 - protein, 16 aa, synthetic construct
  REGION 1..16: note = Chemically Synthesized
  SITE 1: note = MISC_FEATURE - wherein ASN is attached to polyethylene glycol
  SITE 16: note = MISC_FEATURE - wherein LEU is attached to polyethylene glycol
NDECELCVNVACTGCL

SEQ ID NO: 106 - protein, 16 aa, synthetic construct
  REGION 1..16: note = Chemically Synthesized
  SITE 1: note = MISC_FEATURE - wherein ASN is attached to polyethylene glycol
NDECELCVNVACTGCL

SEQ ID NO: 107 - protein, 16 aa, synthetic construct
  REGION 1..16: note = Chemically Synthesized
  SITE 16: note = MISC_FEATURE - wherein LEU is attached to polyethylene glycol
NDECELCVNVACTGCL

SEQ ID NO: 108 - skipped

SEQ ID NO: 109 - protein, 16 aa, synthetic construct
  REGION 1..16: note = Chemically Synthesized
NDDCELCVNVACTGCL

SEQ ID NO: 110 - protein, 16 aa, synthetic construct
  REGION 1..16: note = Chemically Synthesized
EDDCELCVNVACTGCL

SEQ ID NO: 111 - protein, 16 aa, synthetic construct
  REGION 1..16: note = Chemically Synthesized
EDECELCVNVACTGCL

SEQ ID NO: 112 - protein, 16 aa, synthetic construct
  REGION 1..16: note = Chemically Synthesized
EEDCELCVNVACTGCL

SEQ ID NO: 113 - protein, 16 aa, synthetic construct
  REGION 1..16: note = Chemically Synthesized
EEECELCVNVACTGCL

SEQ ID NO: 114 - protein, 16 aa, synthetic construct
  REGION 1..16: note = Chemically Synthesized
DDDCELCVNVACTGCL

SEQ ID NO: 115 - protein, 16 aa, synthetic construct
  REGION 1..16: note = Chemically Synthesized
DDECELCVNVACTGCL

SEQ ID NO: 116 - protein, 16 aa, synthetic construct
  REGION 1..16: note = Chemically Synthesized
DEDCELCVNVACTGCL

SEQ ID NO: 117 - protein, 16 aa, synthetic construct
  REGION 1..16: note = Chemically Synthesized
DEECELCVNVACTGCL

SEQ ID NO: 118 - protein, 16 aa, synthetic construct
  REGION 1..16: note = Chemically Synthesized
QDDCELCVNVACTGCL

SEQ ID NO: 119 - protein, 16 aa, synthetic construct
  REGION 1..16: note = Chemically Synthesized
QDECELCVNVACTGCL

SEQ ID NO: 120 - protein, 16 aa, synthetic construct
  REGION 1..16: note = Chemically Synthesized
QEDCELCVNVACTGCL

SEQ ID NO: 121 - protein, 16 aa, synthetic construct
  REGION 1..16: note = Chemically Synthesized
QEECELCVNVACTGCL

SEQ ID NO: 122 - protein, 16 aa, synthetic construct
  REGION 1..16: note = Chemically Synthesized
KDDCELCVNVACTGCL

SEQ ID NO: 123 - protein, 16 aa, synthetic construct
  REGION 1..16: note = Chemically Synthesized
KDECELCVNVACTGCL

SEQ ID NO: 124 - protein, 16 aa, synthetic construct
  REGION 1..16: note = Chemically Synthesized
KEDCELCVNVACTGCL

SEQ ID NO: 125 - protein, 16 aa, synthetic construct
  REGION 1..16: note = Chemically Synthesized
KEECELCVNVACTGCL

SEQ ID NO: 126 - protein, 16 aa, synthetic construct
  REGION 1..16: note = Chemically Synthesized
EDDCELCVNVACTGCS

SEQ ID NO: 127 - protein, 16 aa, synthetic construct
  REGION 1..16: note = Chemically Synthesized
EDECELCVNVACTGCS

SEQ ID NO: 128 - protein, 16 aa, synthetic construct
  REGION 1..16: note = Chemically Synthesized
EEDCELCVNVACTGCS

SEQ ID NO: 129 - protein, 16 aa, synthetic construct
  REGION 1..16: note = Chemically Synthesized
EEECELCVNVACTGCS

SEQ ID NO: 130 - protein, 16 aa, synthetic construct
  REGION 1..16: note = Chemically Synthesized
DDDCELCVNVACTGCS

SEQ ID NO: 131 - protein, 16 aa, synthetic construct
  REGION 1..16: note = Chemically Synthesized
DDECELCVNVACTGCS

SEQ ID NO: 132 - protein, 16 aa, synthetic construct
  REGION 1..16: note = Chemically Synthesized
DEDCELCVNVACTGCS

SEQ ID NO: 133 - protein, 16 aa, synthetic construct
  REGION 1..16: note = Chemically Synthesized
DEECELCVNVACTGCS

SEQ ID NO: 134 - protein, 16 aa, synthetic construct
  REGION 1..16: note = Chemically Synthesized
QDDCELCVNVACTGCS

SEQ ID NO: 135 - protein, 16 aa, synthetic construct
  REGION 1..16: note = Chemically Synthesized
QDECELCVNVACTGCS

SEQ ID NO: 136 - protein, 16 aa, synthetic construct
  REGION 1..16: note = Chemically Synthesized
QEDCELCVNVACTGCS

SEQ ID NO: 137 - protein, 16 aa, synthetic construct
  REGION 1..16: note = Chemically Synthesized
QEECELCVNVACTGCS

SEQ ID NO: 138 - protein, 16 aa, synthetic construct
  REGION 1..16: note = Chemically Synthesized
KDDCELCVNVACTGCS

SEQ ID NO: 139 - protein, 16 aa, synthetic construct
  REGION 1..16: note = Chemically Synthesized
KDECELCVNVACTGCS

SEQ ID NO: 140 - protein, 16 aa, synthetic construct
  REGION 1..16: note = Chemically Synthesized
KEDCELCVNVACTGCS

SEQ ID NO: 141 - protein, 16 aa, synthetic construct
  REGION 1..16: note = Chemically Synthesized
KEECELCVNVACTGCS

SEQ ID NO: 142 - protein, 16 aa, synthetic construct
  REGION 1..16: note = Chemically Synthesized
EDDCELCINMACTGCL

SEQ ID NO: 143 - protein, 16 aa, synthetic construct
  REGION 1..16: note = Chemically Synthesized
EDECELCINMACTGCL

SEQ ID NO: 144 - protein, 16 aa, synthetic construct
  REGION 1..16: note = Chemically Synthesized
EEDCELCINMACTGCL

SEQ ID NO: 145 - protein, 16 aa, synthetic construct
  REGION 1..16: note = Chemically Synthesized
EEECELCINMACTGCL

SEQ ID NO: 146 - protein, 16 aa, synthetic construct
  REGION 1..16: note = Chemically Synthesized
DDDCELCINMACTGCL

SEQ ID NO: 147 - protein, 16 aa, synthetic construct
  REGION 1..16: note = Chemically Synthesized
DDECELCINMACTGCL

SEQ ID NO: 148 - protein, 16 aa, synthetic construct
  REGION 1..16: note = Chemically Synthesized
DEDCELCINMACTGCL

SEQ ID NO: 149 - protein, 16 aa, synthetic construct
  REGION 1..16: note = Chemically Synthesized
DEECELCINMACTGCL

SEQ ID NO: 150 - protein, 16 aa, synthetic construct
  REGION 1..16: note = Chemically Synthesized
QDDCELCINMACTGCL

SEQ ID NO: 151 - protein, 16 aa, synthetic construct
  REGION 1..16: note = Chemically Synthesized
QDECELCINMACTGCL

SEQ ID NO: 152 - protein, 16 aa, synthetic construct
  REGION 1..16: note = Chemically Synthesized
QEDCELCINMACTGCL

SEQ ID NO: 153 - protein, 16 aa, synthetic construct
  REGION 1..16: note = Chemically Synthesized
QEECELCINMACTGCL

SEQ ID NO: 154 - protein, 16 aa, synthetic construct
  REGION 1..16: note = Chemically Synthesized
KDDCELCINMACTGCL

SEQ ID NO: 155 - protein, 16 aa, synthetic construct
  REGION 1..16: note = Chemically Synthesized
KDECELCINMACTGCL

SEQ ID NO: 156 - protein, 16 aa, synthetic construct
  REGION 1..16: note = Chemically Synthesized
KEDCELCINMACTGCL

SEQ ID NO: 157 - protein, 16 aa, synthetic construct
  REGION 1..16: note = Chemically Synthesized
KEECELCINMACTGCL

SEQ ID NO: 158 - protein, 16 aa, synthetic construct
  REGION 1..16: note = Chemically Synthesized
EDDCELCINMACTGCS

SEQ ID NO: 159 - protein, 16 aa, synthetic construct
  REGION 1..16: note = Chemically Synthesized
EDECELCINMACTGCS

SEQ ID NO: 160 - protein, 16 aa, synthetic construct
  REGION 1..16: note = Chemically Synthesized
EEDCELCINMACTGCS

SEQ ID NO: 161 - protein, 16 aa, synthetic construct
  REGION 1..16: note = Chemically Synthesized
EEECELCINMACTGCS

SEQ ID NO: 162 - protein, 16 aa, synthetic construct
  REGION 1..16: note = Chemically Synthesized
DDDCELCINMACTGCS

SEQ ID NO: 163 - protein, 16 aa, synthetic construct
  REGION 1..16: note = Chemically Synthesized
DDECELCINMACTGCS

SEQ ID NO: 164 - protein, 16 aa, synthetic construct
  REGION 1..16: note = Chemically Synthesized
DEDCELCINMACTGCS

SEQ ID NO: 165 - protein, 16 aa, synthetic construct
  REGION 1..16: note = Chemically Synthesized
DEECELCINMACTGCS

SEQ ID NO: 166 - protein, 16 aa, synthetic construct
  REGION 1..16: note = Chemically Synthesized
QDDCELCINMACTGCS

SEQ ID NO: 167 - protein, 16 aa, synthetic construct
  REGION 1..16: note = Chemically Synthesized
QDECELCINMACTGCS

SEQ ID NO: 168 - protein, 16 aa, synthetic construct
  REGION 1..16: note = Chemically Synthesized
QEDCELCINMACTGCS

SEQ ID NO: 169 - protein, 16 aa, synthetic construct
  REGION 1..16: note = Chemically Synthesized
QEECELCINMACTGCS

SEQ ID NO: 170 - protein, 16 aa, synthetic construct
  REGION 1..16: note = Chemically Synthesized
KDDCELCINMACTGCS

SEQ ID NO: 171 - protein, 16 aa, synthetic construct
  REGION 1..16: note = Chemically Synthesized
KDECELCINMACTGCS

SEQ ID NO: 172 - protein, 16 aa, synthetic construct
  REGION 1..16: note = Chemically Synthesized
KEDCELCINMACTGCS

SEQ ID NO: 173 - protein, 16 aa, synthetic construct
  REGION 1..16: note = Chemically Synthesized
KEECELCINMACTGCS

SEQ ID NO: 174 - skipped

SEQ ID NO: 175 - protein, 15 aa, synthetic construct
  REGION 1..15: note = Chemically Synthesized
SHTCEICAFAACAGC

SEQ ID NO: 176 - protein, 15 aa, synthetic construct
  REGION 1..15: note = Chemically Synthesized
SHTCEICANAACAGC

SEQ ID NO: 177 - protein, 15 aa, synthetic construct
  REGION 1..15: note = Chemically Synthesized
SHTCELCANAACAGC

SEQ ID NO: 178 - protein, 15 aa, synthetic construct
  REGION 1..15: note = Chemically Synthesized
SHTCEVCANAACAGC

SEQ ID NO: 179 - protein, 15 aa, synthetic construct
  REGION 1..15: note = Chemically Synthesized
SHTCEYCANAACAGC

SEQ ID NO: 180 - protein, 15 aa, synthetic construct
  REGION 1..15: note = Chemically Synthesized
SHTCEICANAACAGC

SEQ ID NO: 181 - protein, 15 aa, synthetic construct
  REGION 1..15: note = Chemically Synthesized
SHTCELCANAACAGC

SEQ ID NO: 182 - protein, 15 aa, synthetic construct
  REGION 1..15: note = Chemically Synthesized
SHTCEVCANAACAGC

SEQ ID NO: 183 - protein, 15 aa, synthetic construct
  REGION 1..15: note = Chemically Synthesized
SHTCEYCANAACAGC

SEQ ID NO: 184 - protein, 15 aa, synthetic construct
  REGION 1..15: note = Chemically Synthesized
SHTCEICANAACAGC

SEQ ID NO: 185 - protein, 15 aa, synthetic construct
  REGION 1..15: note = Chemically Synthesized
SHTCELCANAACAGC

SEQ ID NO: 186 - protein, 15 aa, synthetic construct
  REGION 1..15: note = Chemically Synthesized
SHTCEVCANAACAGC

SEQ ID NO: 187 - protein, 15 aa, synthetic construct
  REGION 1..15: note = Chemically Synthesized
SHTCEYCANAACAGC

SEQ ID NO: 188 - protein, 15 aa, synthetic construct
  REGION 1..15: note = Chemically Synthesized
SHTCEICANAACAGC

SEQ ID NO: 189 - protein, 15 aa, synthetic construct
  REGION 1..15: note = Chemically Synthesized
SHTCELCANAACAGC

SEQ ID NO: 190 - protein, 15 aa, synthetic construct
  REGION 1..15: note = Chemically Synthesized
SHTCEVCANAACAGC

SEQ ID NO: 191 - protein, 15 aa, synthetic construct
  REGION 1..15: note = Chemically Synthesized
SHTCEYCANAACAGC

SEQ ID NO: 192 - protein, 15 aa, synthetic construct
  REGION 1..15: note = Chemically Synthesized
NDECEICANAACAGC

SEQ ID NO: 193 - protein, 15 aa, synthetic construct
  REGION 1..15: note = Chemically Synthesized
NDECELCANAACAGC

SEQ ID NO: 194 - protein, 15 aa, synthetic construct
  REGION 1..15: note = Chemically Synthesized
NDECEVCANAACAGC

SEQ ID NO: 195 - protein, 15 aa, synthetic construct
  REGION 1..15: note = Chemically Synthesized
NDECEYCANAACAGC

SEQ ID NO: 196 - protein, 15 aa, synthetic construct
  REGION 1..15: note = Chemically Synthesized
NDECEICANAACAGC

SEQ ID NO: 197 - protein, 15 aa, synthetic construct
  REGION 1..15: note = Chemically Synthesized
NDECELCANAACAGC

SEQ ID NO: 198 - protein, 15 aa, synthetic construct
  REGION 1..15: note = Chemically Synthesized
NDECEVCANAACAGC

SEQ ID NO: 199 - protein, 15 aa, synthetic construct
  REGION 1..15: note = Chemically Synthesized
NDECEYCANAACAGC

SEQ ID NO: 200 - protein, 15 aa, synthetic construct
  REGION 1..15: note = Chemically Synthesized
NDECEICANAACAGC

SEQ ID NO: 201 - protein, 15 aa, synthetic construct
  REGION 1..15: note = Chemically Synthesized
NDECELCANAACAGC

SEQ ID NO: 202 - protein, 15 aa, synthetic construct
  REGION 1..15: note = Chemically Synthesized
NDECEVCANAACAGC

SEQ ID NO: 203 - protein, 15 aa, synthetic construct
  REGION 1..15: note = Chemically Synthesized
NDECEYCANAACAGC

SEQ ID NO: 204 - protein, 15 aa, synthetic construct
  REGION 1..15: note = Chemically Synthesized
NDECEICANAACAGC

SEQ ID NO: 205 - protein, 15 aa, synthetic construct
  REGION 1..15: note = Chemically Synthesized
NDECELCANAACAGC

SEQ ID NO: 206 - protein, 15 aa, synthetic construct
  REGION 1..15: note = Chemically Synthesized
NDECEVCANAACAGC

SEQ ID NO: 207 - protein, 15 aa, synthetic construct
  REGION 1..15: note = Chemically Synthesized
NDECEYCANAACAGC

SEQ ID NO: 208 - skipped

SEQ ID NO: 209 - protein, 15 aa, synthetic construct
  REGION 1..15: note = Chemically Synthesized
QEECELCINMACTGY

SEQ ID NO: 210 - protein, 15 aa, synthetic construct
  REGION 1..15: note = Chemically Synthesized
QEECETCINMACTGY

SEQ ID NO: 211 - protein, 15 aa, synthetic construct
  REGION 1..15: note = Chemically Synthesized
QDECETCINMACTGY

SEQ ID NO: 212 - protein, 15 aa, synthetic construct
  REGION 1..15: note = Chemically Synthesized
QDDCETCINMACTGY

SEQ ID NO: 213 - protein, 15 aa, synthetic construct
  REGION 1..15: note = Chemically Synthesized
QEDCETCINMACTGY

SEQ ID NO: 214 - protein, 15 aa, synthetic construct
  REGION 1..15: note = Chemically Synthesized
QEECEECINMACTGY

SEQ ID NO: 215 - protein, 15 aa, synthetic construct
  REGION 1..15: note = Chemically Synthesized
QDECEECINMACTGY

SEQ ID NO: 216 - protein, 15 aa, synthetic construct
  REGION 1..15: note = Chemically Synthesized
QDDCEECINMACTGY

SEQ ID NO: 217 - protein, 15 aa, synthetic construct
  REGION 1..15: note = Chemically Synthesized
QEDCEECINMACTGY

SEQ ID NO: 218 - protein, 15 aa, synthetic construct
  REGION 1..15: note = Chemically Synthesized
QEECEYCINMACTGY

SEQ ID NO: 219 - protein, 15 aa, synthetic construct
  REGION 1..15: note = Chemically Synthesized
QDECEYCINMACTGY

SEQ ID NO: 220 - protein, 15 aa, synthetic construct
  REGION 1..15: note = Chemically Synthesized
QDDCEYCINMACTGY

SEQ ID NO: 221 - protein, 15 aa, synthetic construct
  REGION 1..15: note = Chemically Synthesized
QEDCEYCINMACTGY

SEQ ID NO: 222 - protein, 15 aa, synthetic construct
  REGION 1..15: note = Chemically Synthesized
QEECEICINMACTGY

SEQ ID NO: 223 - protein, 15 aa, synthetic construct
  REGION 1..15: note = Chemically Synthesized
QDECEICINMACTGY

SEQ ID NO: 224 - protein, 15 aa, synthetic construct
  REGION 1..15: note = Chemically Synthesized
QDDCEICINMACTGY

SEQ ID NO: 225 - protein, 15 aa, synthetic construct
  REGION 1..15: note = Chemically Synthesized
QEDCEICINMACTGY

SEQ ID NO: 226 - protein, 16 aa, synthetic construct
  REGION 1..16: note = Chemically Synthesized
QEECETCINMACTGCS

SEQ ID NO: 227 - protein, 16 aa, synthetic construct
  REGION 1..16: note = Chemically Synthesized
QDECETCINMACTGCS

SEQ ID NO: 228 - protein, 16 aa, synthetic construct
  REGION 1..16: note = Chemically Synthesized
QDDCETCINMACTGCS

SEQ ID NO: 229 - protein, 16 aa, synthetic construct
  REGION 1..16: note = Chemically Synthesized
QEDCETCINMACTGCS

SEQ ID NO: 230 - protein, 16 aa, synthetic construct
  REGION 1..16: note = Chemically Synthesized
QEECEECINMACTGCS

SEQ ID NO: 231 - protein, 16 aa, synthetic construct
  REGION 1..16: note = Chemically Synthesized
QDECEECINMACTGCS

SEQ ID NO: 232 - protein, 16 aa, synthetic construct
  REGION 1..16: note = Chemically Synthesized
QDDCEECINMACTGCS

SEQ ID NO: 233 - protein, 16 aa, synthetic construct
  REGION 1..16: note = Chemically Synthesized
QEDCEECINMACTGCS

SEQ ID NO: 234 - protein, 16 aa, synthetic construct
  REGION 1..16: note = Chemically Synthesized
QEECEYCINMACTGCS

SEQ ID NO: 235 - protein, 16 aa, synthetic construct
  REGION 1..16: note = Chemically Synthesized
QDECEYCINMACTGCS

SEQ ID NO: 236 - protein, 16 aa, synthetic construct
  REGION 1..16: note = Chemically Synthesized
QDDCEYCINMACTGCS

SEQ ID NO: 237 - protein, 16 aa, synthetic construct
  REGION 1..16: note = Chemically Synthesized
QEDCEYCINMACTGCS

SEQ ID NO: 238 - protein, 16 aa, synthetic construct
  REGION 1..16: note = Chemically Synthesized
QEECEICINMACTGCS

SEQ ID NO: 239 - protein, 16 aa, synthetic construct
  REGION 1..16: note = Chemically Synthesized
QDECEICINMACTGCS

SEQ ID NO: 240 - protein, 16 aa, synthetic construct
  REGION 1..16: note = Chemically Synthesized
QDDCEICINMACTGCS

SEQ ID NO: 241 - protein, 16 aa, synthetic construct
  REGION 1..16: note = Chemically Synthesized
QEDCEICINMACTGCS

SEQ ID NO: 242 - protein, 22 aa, synthetic construct
  REGION 1..22: note = Chemically Synthesized
NSSNSSNYCCEKCCNPACTGCY

SEQ ID NO: 243 - protein, 16 aa, synthetic construct
  REGION 1..16: note = Chemically Synthesized
  SITE 1: note = MISC_FEATURE - wherein ASN is attached to polyethylene glycol
  SITE 16: note = MISC_FEATURE - wherein TYR is attached to polyethylene glycol
NFCCETCCNPACTGCY

SEQ ID NO: 244 - protein, 16 aa, synthetic construct
  REGION 1..16: note = Chemically Synthesized
  SITE 1: note = MISC_FEATURE - wherein ASN is attached to polyethylene glycol
NFCCETCCNPACTGCY

SEQ ID NO: 245 - protein, 16 aa, synthetic construct
  REGION 1..16: note = Chemically Synthesized
  SITE 16: note = MISC_FEATURE - wherein TYR is attached to polyethylene glycol
NFCCETCCNPACTGCY

SEQ ID NO: 246 - protein, 16 aa, synthetic construct
  REGION 1..16: note = Chemically Synthesized
NFCCEYCCNPACTGCY

SEQ ID NO: 247 - protein, 16 aa, synthetic construct
  REGION 1..16: note = Chemically Synthesized
  SITE 1: note = MISC_FEATURE - wherein ASN is a D amino acid
  SITE 16: note = MISC_FEATURE - wherein TYR is a D amino acid
NFCCEYCCNPACTGCY

SEQ ID NO: 248 - protein, 16 aa, synthetic construct
  REGION 1..16: note = Chemically Synthesized
  SITE 16: note = MISC_FEATURE - wherein TYR is a D amino acid
NFCCEYCCNPACTGCY

SEQ ID NO: 249 - protein, 16 aa, synthetic construct
  REGION 1..16: note = Chemically Synthesized
  SITE 1: note = MISC_FEATURE - wherein ASN is a D amino acid
NFCCEYCCNPACTGCY

SEQ ID NO: 250 - skipped

SEQ ID NO: 251 - protein, 16 aa, synthetic construct
  REGION 1..16: note = Synthesized peptide
  SITE 1: note = MISC_FEATURE - wherein Xaa is a pyroglutamic acid
XDECELCVNVACTGCL

SEQ ID NO: 252 - protein, 15 aa, synthetic construct
  REGION 1..15: note = Synthesized peptide
PGTCEICAYAACTGC